European Patent Application EP 4 756 033 A1, published June 10, 2026. Title: Biosynthesis of Indigo Dyestuff with Tunable Color Hue. Applicant: Nano and Advanced Materials Institute Limited. Application EP. The sequence listing filed with the application follows.

SEQUENCE LISTING (2 sequences)

SEQ ID NO: 1 - DNA, 1417 bp, synthetic construct
  source 1..1417: mol_type = other DNA
atggagaactttaagcatttacctgagccattccggatccgtgttattgagccagttaaacggacaacccgagcatatcgtgaagaagcgatcataaaatcaggtatgaatccttttttgctggatagcgaagatgtttttattgacttgctgacagattccggtacaggagccgttacgcaaagtatgcaggctgcgatgatgagaggcgacgaggcgtacagcggttctcgttcgtactatgcccttgcagagagtgttaaaaatatttttggttatcaatacaccataccgacgcaccaaggacgcggggcagaacaaatctatatacccgtgttgatcaaaaagcgcgaacaggaaaagggactcgatcgatccaaaatggtggccttttccaattatttttttgacaccactcaaggtcattcccagattaacggctgtaccgtgcggaatgtatatattaaagaagcattcgatactggggtgcgttatgactttaaaggcaatttcgatctggagggtttagaacgcggcatagaagaagttgggccaaataatgttccttacatcgttgcaaccattacctcaaatagtgcgggtggccaacctgtttcattagcgaacctcaaagccatgtattccattgcgaaaaaatatgatattcctgtggtgatggattccgcaagattcgcggaaaatgcgtatttcataaaacagcgcgaggctgaatataaagactggacaattgaacaaatcacacgtgaaacgtataaatatgctgacatgcttgctatgagcgcgaaaaaagatgcgatggtccctatgggggggcttctgtgtatgaaagatgattcgttttttgacgtttacacggagtgtcgtacgctttgtgtagtacaagaaggctttccaacatatggcggcctcgaagggggcgcaatggaacgtcttgcagttggcctttatgatggaatgaatttagattggctggcataccgtattgcccaggtccagtatctggtggatggcctcgaagaaatcggcgttgtgtgtcagcaggccggtggtcacgccgcatttgttgatgccggcaaactgcttccgcacatcccggcagaccaatttcctgcgcaggcactggcgtgcgaactgtataaggtggcgggtatccgcgccgtggagataggcagttttcttcttgggcgtgatccgaaaaccgggaaacaactgccatgcccagcggaactgctgcgcctcacgataccgcgtgcgacatatacccaaacccatatggatttcatcattgaagcgtttaaacatgtgaaagaaaatgccgcgaacattaaaggcttaacttttacctatgagccaaaagttctgcggcactttacagcaaaattgaaagaagtttaac

SEQ ID NO: 2 - DNA, 1371 bp, synthetic construct
  source 1..1371: mol_type = other DNA
atggcaactcgaattgcaattttaggtgctgggccaagcggcatggcgcagctgcgcgcgttccagtctgcccaagaaaaaggcgcagaaattcctgagttggtgtgcttcgaaaaacaggccgactggggtggccaatggaattatacatggagaacagggttggacgaaaacggtgagcctgttcactcttcgatgtaccgttacctgtggtctaacggaccaaaagagtgcctcgaatttgccgactacacctttgatgagcatttcggcaaacctattgcatcgtatccaccgagagaagttttatgggactatataaaaggtcgcgtagagaaggcaggcgttcggaaatacattagatttaatactgcggtgcgccacgtcgaattcaacgaagattcccaaacatttacggtgacagtacaggatcatactacagacaccatttattcagaggaatttgattatgtggtctgctgtaccggccactttagcacgccttacgtgcctgaatttgaaggttttgagaaatttggtggtcgaattctgcatgcgcatgatttccgggatgctttagagttcaaagataagacggtactgctggttggttcatcctactctgcggaagatatagggtcacagtgctataagtatggggcaaaaaagctgattagttgttaccgcaccgcacctatgggatataaatggccggaaaactgggatgagcgtcctaatttagttcgtgtagatacggaaaatgcatatttcgctgatggctcatctgaaaaagtggacgctataatcctctgcacgggttatattcatcactttccattcctgaacgacgacctgcgcttggtgacaaacaatcgtctgtggccgctcaacctgtataaaggtgtggtctgggaagataatcctaaatttttttatatagggatgcaggatcagtggtattcttttaatatgtttgacgcccaggcatggtatgcgcgagatgttattatgggacgtctcccgcttccgagtaaagaggaaatgaaagctgactcaatggcttggcgcgaaaaagaactgactttggtcacggcggaagagatgtatacttatcaaggcgattacatccagaatcttattgatatgacagactatccgtcttttgatattcccgcaaccaacaaaacctttttggaatggaaacatcacaaaaaagaaaatattatgacgttccgtgatcatagctaccgcagccttatgactggcacaatggcccctaagcatcatactccctggattgatgccctggatgattctttggaagcgtatctctccgataaatcggaaatcccagttgccaaggaggcataa